European Patent Specification EP 3 958 890 B1, published November 20, 2024. Title: Beta-Amylase Variants. Applicant: BASF SE. The sequence listing filed with the application follows.

SEQUENCE LISTING (3 sequences)

SEQ ID NO: 1 - protein, 519 aa, Clostridium Thermosulfurogenes
SIAPNFKVFVMGPLEKVTDFNAFKDQLITLKNNGVYGITTDIWWGYVENAGENQFDWSYYKTYADTVRAAGLKWVPIMSTHACGGNVGDTVNIPIPSWVWTKDTQDNMQYKDEAGNWDNEAVSPWYSGLTQLYNEFYSSFASNFSSYKDIITKIYISGGPSGELRYPSYNPSHGWTYPGRGSLQCYSKAAITSFQNAMKSKYGTIAAVNSAWGTSLTDFSQISPPTDGDNFFTNGYKTTYGNDFLTWYQSVLTNELANIASVAHSCFDPVFNVPIGAKIAGVHWLYNSPTMPHAAEYCAGYYNYSTLLDQFKASNLAMTFTCLEMDDSNAYVSPYYSAPMTLVHYVANLANNKGIVHNGENALAISNNNQAYVNCANELTGYNFSGFTLLRLSNIVNSDGSVTSEMAPFVINIVTLTPNGTIPVTFTINNATTYYGQNVYIVGSTSDLGNWNTTYARGPASCPNYPTWTITLNLLPGEQIQFKAVKIDSSGNVTWEGGSNHTYTVPTSGTGSVTITWQN

SEQ ID NO: 2 - protein, 519 aa, Artificial Sequence
  Synthetic generation
SIAPNFKVFVMGPLEKVTDFNAFKKQCITLKNNGVYGITTDIWWGYVENAGENQFDWSYYKTYADTVRAAGLKWVPIMSTHACGGNVGDTVNIPIPSWVWTKDTQDNMQYKDEAGNWDNEAVSPWYSGLTQLYNEFYSSFASNFSSYKDIITKIYISGGPSGELRYPSYNPSHGWTYPGRGSLQCYSKAAITSFQNAMKSKYGTIAAVNSAWGTSLTDFLQISPPTDGDNFFTNGYKTTYGNDFLTWYQSVLTNELANIASVAHSCFDPVFNVPIGAKIAGVHWLYNSPTMPHAAEYCAGYYNYSTLLDQFKASNLAMTFTCLEMDDSNAYVSPYYSAPMTLVHYVANLANNKGIVHNGENALPISNNPQAYVNCANELTGYNFSGFTLLRLSNIVNPDGSVTSEMAPFVINIVTLTPNGTIPVTFTINNATTYYGQNVYIVGSTSDLGNWNTTYARGPASCPNYPTWTITLNLLPGEQIQFKAVKIDSSGNVTWEGGSNHTYTVPTSGTGSVTITWQN

SEQ ID NO: 3 - protein, 519 aa, Artificial Sequence
  Synthetic Generation
SIAPNFKVFVMGPLEKVTDFNAFKKQCITLKNNGVYGITTDIWWGYVENAGENQFDWSYYKTYADTVRAAGLKWVPIMSTHACGGNVGDTVNIPIPSWVWTKDTQDNMQYKDEAGNWDNEAVSPWYSGLTQLYNEFYSSFASNFSSYKDIITKIYISGGPSGELRYPSYNPSHGWTYPGRGSLQCYSKAAITSFQNAMKSKYGTIAAVNSAWGTSLTDFLQISPPTDGDNFFTNGYKTTYGNDFLTWYQSVLTNELANIASVAHSCFDPVFNVPIGAKIAGVHWLYNSPTMPHAAEYCAGYYNYSTLLDQFKASNLAMTFTCLEMDDSNAYVSPYYSAPMTLVHYVANLANNKGIVHNGENALPISNNPQAYVNCANELTGYNFSGFTLLRLSNIVNPDGSVTSEMAPFVINIVTLTPEGTIPVTFTINNATTYYGQNVYIVGSTSDLGNWNTTYARGPASCPNYPTWTITLNLLPGEQIQFKAVKIDSSGNVEWEGGSNHEYTVPTSGTGSVTITWQN